European Patent Application EP 4 386 090 A1, published June 19, 2024. Title: Method for determining and improving the potential efficacy of anticancer treatment. Applicant: ASSISTANCE PUBLIQUE - HOPITAUX DE PARIS. Application EP. The sequence listing filed with the application follows.

SEQUENCE LISTING (5 sequences)

SEQ ID NO: 1 - DNA, 454 bp, Bacteroides fragilis
  source 1..454: mol_type = genomic DNA
acgggaggcagcagtgaggaatattggtcaatgggcgctagcctgaaccagccaagtagcgtgaaggatgaaggctctatgggtcgtaaacttcttttatataagaataaagtgcagtatgtatactgttttgtatgtattatatgaataaggatcggctaactccgtgccagcagccgcggtaatacggaggatccgagcgttatccggatttattgggtttaaagggagcgtaggtggactggtaagtcagttgtgaaagtttgcggctcaaccgtaaaattgcagttgatactgtcagtcttgagtacagtagaggtgggcggaattcgtggtgtagcggtgaaatgcttagatatcacgaagaactccgattgcgaaggcagctcactggactgcaactgacactgatgctcgaaagtgtgggtatcaaacaggattagataccctggta

SEQ ID NO: 2 - DNA, 454 bp, Bacteroides sp. DJF_B097
  source 1..454: mol_type = genomic DNA
acgggaggcagcagtgaggaatattggtcaatggacgagagtctgaaccagccaagtagcgtgaaggatgactgccctatgggttgtaaacttcttttatacgggaataaagttagccacgtgtggctttttgtatgtaccgtatgaataaggatcggctaactccgtgccagcagccgcggtaatacggaggatccgagcgttatccggatttattgggtttaaagggagcgtaggcgggttgttaagtcagttgtgaaagtttgcggctcaaccgtaaaattgcagttgatactggcgaccttgagtgcaacagaggtaggcggaattcgtggtgtagcggtgaaatgcttagatatcacgaagaactccgattgcgaaggcagcttactggattgtaactgacgctgatgctcgaaagtgtgggtatcaaacaggattagataccctggta

SEQ ID NO: 3 - DNA, 454 bp, Prevotella sp. DJF_RP53
  source 1..454: mol_type = genomic DNA
acgggaggcagcagtgaggaatattggtcaatggacgagagtctgaaccagccaagtagcgtgcaggaagacggccctatgggttgtaaactgcttttataagggaataaagtgagagtcgtgactctttttgcatgtaccttatgaataaggaccggctaattccgtgccagcagccgcggtaatacggaaggtccgggcgttatccggatttattgggtttaaagggagcgtaggccggagattaagcgtgttgtgaaatgtagatgctcaacatctgaactgcagcgcgaactggtttccttgagtacgcacaaagtgggcggaattcgtggtgtagcggtgaaatgcttagatatcacgaagaactccgattgcgaaggcagctcactggagcgcaactgacgctgaagctcgaaagtgcgggtatcgaacaggattagataccctggta

SEQ ID NO: 4 - DNA, 15 bp, synthetic construct
  source 1..15: mol_type = other DNA
tacggraggcagcag

SEQ ID NO: 5 - DNA, 16 bp, synthetic construct
  source 1..16: mol_type = other DNA
taccagggtatctaat